European Patent Application EP 4 806 912 A1, published September 16, 2026. Title: DUAL AGONIST COMPOUND. Applicant: Chengdu Aoda Biotechnology CO.,Ltd. The sequence listing filed with the application follows.

SEQUENCE LISTING (16 sequences)

SEQ ID NO: 1 - protein, 34 aa, synthetic construct
  MOD_RES 2: note = X is Aib
  MOD_RES 20: note = X is Lys(2-(2-aminoethoxy) ethoxyacetic acid-gamma Glu-eicosanedioic acid)
HXQGTFTSDYSKYLDEKKAXEFVEWLLEGGPSSG

SEQ ID NO: 2 - protein, 38 aa, synthetic construct
  MOD_RES 2: note = X is Aib
  MOD_RES 20: note = X is Lys(COCH2PEG5-Gamma Glu-eicosanedioic acid)
  MOD_RES 29: note = X is 5-Ava
HXQGTFTSDYSKYLDEKKAXEFVEWLLEXPSSGAPPPS

SEQ ID NO: 3 - protein, 38 aa, synthetic construct; identical to SEQ ID NO: 2
  MOD_RES 2: note = X is Aib
  MOD_RES 20: note = X is Lys(COCH2PEG5-Delta Aad-eicosanedioic acid)
  MOD_RES 29: note = X is 5-Ava

SEQ ID NO: 4 - protein, 38 aa, synthetic construct; identical to SEQ ID NO: 2
  MOD_RES 2: note = X is Aib
  MOD_RES 20: note = X is Lys(COCH2PEG5-Epsilon Apm-eicosanedioic acid)
  MOD_RES 29: note = X is 5-Ava

SEQ ID NO: 5 - protein, 38 aa, synthetic construct; identical to SEQ ID NO: 2
  MOD_RES 2: note = X is Aib
  MOD_RES 20: note = X is Lys(COCH2PEG5-Zeta Asu-eicosanedioic acid)
  MOD_RES 29: note = X is 5-Ava

SEQ ID NO: 6 - protein, 38 aa, synthetic construct
  MOD_RES 2: note = X is Aib
  MOD_RES 6: note = X is alpha-MePhe
  MOD_RES 20: note = X is Lys(PEG5CH2CO-Gamma Glu-eicosanedioic acid)
  MOD_RES 29: note = X is 5-Ava
HXQGTXTSDYSKYLDEKKAXEFVEWLLEXPSSGAPPPS

SEQ ID NO: 7 - protein, 38 aa, synthetic construct; identical to SEQ ID NO: 6
  MOD_RES 2: note = X is Aib
  MOD_RES 6: note = X is alpha-MePhe
  MOD_RES 20: note = X is Lys(COCH2PEG5-Delta Aad-eicosanedioic acid)
  MOD_RES 29: note = X is 5-Ava

SEQ ID NO: 8 - protein, 38 aa, synthetic construct; identical to SEQ ID NO: 6
  MOD_RES 2: note = X is Aib
  MOD_RES 6: note = X is alpha-MePhe
  MOD_RES 20: note = X is Lys(COCH2PEG5-Epsilon Apm-eicosanedioic acid)
  MOD_RES 29: note = X is 5-Ava

SEQ ID NO: 9 - protein, 38 aa, synthetic construct; identical to SEQ ID NO: 6
  MOD_RES 2: note = X is Aib
  MOD_RES 6: note = X is alpha-MePhe
  MOD_RES 20: note = X is Lys(COCH2PEG5-Zeta Asu-eicosanedioic acid)
  MOD_RES 29: note = X is 5-Ava

SEQ ID NO: 10 - protein, 38 aa, synthetic construct; identical to SEQ ID NO: 6
  MOD_RES 2: note = X is Aib
  MOD_RES 6: note = X is alpha-MePhe(2F)
  MOD_RES 20: note = X is Lys(PEG5CH2CO-Gamma Glu-eicosanedioic acid)
  MOD_RES 29: note = X is 5-Ava

SEQ ID NO: 11 - protein, 38 aa, synthetic construct; identical to SEQ ID NO: 6
  MOD_RES 2: note = X is Aib
  MOD_RES 6: note = X is alpha-MePhe(2F)
  MOD_RES 20: note = X is Lys(COCH2PEG5-Delta Aad-eicosanedioic acid)
  MOD_RES 29: note = X is 5-Ava

SEQ ID NO: 12 - protein, 38 aa, synthetic construct; identical to SEQ ID NO: 6
  MOD_RES 2: note = X is Aib
  MOD_RES 6: note = X is alpha-MePhe(2F)
  MOD_RES 20: note = X is Lys(COCH2PEG5-Epsilon Apm-eicosanedioic acid)
  MOD_RES 29: note = X is 5-Ava

SEQ ID NO: 13 - protein, 38 aa, synthetic construct; identical to SEQ ID NO: 6
  MOD_RES 2: note = X is Aib
  MOD_RES 6: note = X is alpha-MePhe(2F)
  MOD_RES 20: note = X is Lys(COCH2PEG5-Zeta Asu-eicosanedioic acid)
  MOD_RES 29: note = X is 5-Ava

SEQ ID NO: 14 - protein, 38 aa, synthetic construct; identical to SEQ ID NO: 2
  MOD_RES 2: note = X is Aib
  MOD_RES 20: note = X is Lys(2-(2-aminoethoxy) ethoxyacetic acid-2-(2-aminoethoxy) ethoxyacetic acid-Gamma Glu-eicosanedioic acid)
  MOD_RES 29: note = X is 5-Ava

SEQ ID NO: 15 - protein, 38 aa, synthetic construct; identical to SEQ ID NO: 6
  MOD_RES 2: note = X is Aib
  MOD_RES 6: note = X is alpha-MePhe
  MOD_RES 20: note = X is Lys(2-(2-aminoethoxy) ethoxyacetic acid-2-(2-aminoethoxy) ethoxyacetic acid-Gamma Glu-eicosanedioic acid)
  MOD_RES 29: note = X is 5-Ava

SEQ ID NO: 16 - protein, 38 aa, synthetic construct; identical to SEQ ID NO: 6
  MOD_RES 2: note = X is Aib
  MOD_RES 6: note = X is alpha-MePhe(2F)
  MOD_RES 20: note = X is Lys(2-(2-aminoethoxy) ethoxyacetic acid-2-(2-aminoethoxy) ethoxyacetic acid-Gamma Glu-eicosanedioic acid)
  MOD_RES 29: note = X is 5-Ava